European Patent Specification EP 3 674 318 B1, published November 27, 2024. Title: Optimized Fc variants. Applicant: LABORATOIRE FRANÇAIS DU FRACTIONNEMENT ET DES BIOTECHNOLOGIES. The sequence listing filed with the application follows.

SEQUENCE LISTING (16 sequences)

SEQ ID NO: 1 - protein, 222 aa, Homo sapiens
  MISC_FEATURE (131)..(131): For G1m1,17 allotype, X is D
  MISC_FEATURE (131)..(131): For G1m3 allotype, X is E
  MISC_FEATURE (133)..(133): For G1m1,17 allotype, X is L
  MISC_FEATURE (133)..(133): For G1m3 allotype, X is M
CPPCPAPELLGGPSVFLFPPKPKDTLMISRTPEVTCVVVDVSHEDPEVKFNWYVDGVEVHNAKTKPREEQYNSTYRVVSVLTVLHQDWLNGKEYKCKVSNKALPAPIEKTISKAKGQPREPQVYTLPPSRXEXTKNQVSLTCLVKGFYPSDIAVEWESNGQPENNYKTTPPVLDSDGSFFLYSKLTVDKSRWQQGNVFSCSVMHEALHNHYTQKSLSLSPGK

SEQ ID NO: 2 - protein, 221 aa, Homo sapiens
CPPCPAPPVAGPSVFLFPPKPKDTLMISRTPEVTCVVVDVSHEDPEVQFNWYVDGVEVHNAKTKPREEQYNSTYRVVSVLTVLHQDWLNGKEYKCKVSNKALPAPIEKTISKTKGQPREPQVYTLPPSREEMTKNQVSLTCLVKGFYPSDIAVEWESNGQPENNYKTTPPMLDSDGSFFLYSKLTVDKSRWQQGNVFSCSVMHEALHNHYTQKSLSLSPGK

SEQ ID NO: 3 - protein, 222 aa, Homo sapiens
CPRCPAPELLGGPSVFLFPPKPKDTLMISRTPEVTCVVVDVSHEDPEVQFKWYVDGVEVHNAKTKPREEQYNSTFRVVSVLTVLHQDWLNGKEYKCKVSNKALPAPIEKTISKTKGQPREPQVYTLPPSREEMTKNQVSLTCLVKGFYPSDIAVEWESSGQPENNYNTTPPMLDSDGSFFLYSKLTVDKSRWQQGNIFSCSVMHEALHNRFTQKSLSLSPGK

SEQ ID NO: 4 - protein, 221 aa, Homo sapiens
CPSPAPEFLGGPSVFLFPPKPKDTLMISRTPEVTCVVVDVSQEDPEVQFNWYVDGMEVHNAKTKPREEQFNSTFRVVSVLTVVHQDWLNGKEYKCKVSNKGLPAPIEKTISKAKGQPREPQVYTLPPSQEEMTKNQVSLTCLVKGFYPSDIAVEWESNGQPENNYKTTPPVLDSDGSFFLYSRLTVDKSRWQEGNVFSCSVMHEALHNHYTQKSLSLSLGK

SEQ ID NO: 5 - DNA, 35 bp, Artificial
  Primer
agtactgactctacctaggatcctgcccaccgtgc

SEQ ID NO: 6 - DNA, 35 bp, Artificial
  Primer
actgctcgatgtccgtactatgcggccgcgaattc

SEQ ID NO: 7 - DNA, 18 bp, Artificial
  primer
caggaaacagctatgacc

SEQ ID NO: 8 - DNA, 20 bp, Artificial
  Primer
tcacgtgcaaaagcagcggc

SEQ ID NO: 9 - DNA, 18 bp, Artificial
  Primer
tgattacgccaagcttgc

SEQ ID NO: 10 - DNA, 100 bp, Artificial
  Primer
cgggatcctgcccaccgtgcccagcacctgaactcctggggggaccgtcagtcttcctcttccccccaaaacccaaggaccaactcatgatctcccggac

SEQ ID NO: 11 - DNA, 84 bp, Artificial
  Primer
gcgaattctttacccggagacagggagaggctcttctgcgtgtagtggttgtgcagagcctcatgcagcacggagcatgagaag

SEQ ID NO: 12 - protein, 232 aa, Homo sapiens
EPKSCDKTHTCPPCPAPELLGGPSVFLFPPKPKDTLMISRTPEVTCVVVDVSHEDPEVKFNWYVDGVEVHNAKTKPREEQYNSTYRVVSVLTVLHQDWLNGKEYKCKVSNKALPAPIEKTISKAKGQPREPQVYTLPPSRDELTKNQVSLTCLVKGFYPSDIAVEWESNGQPENNYKTTPPVLDSDGSFFLYSKLTVDKSRWQQGNVFSCSVMHEALHNHYTQKSLSLSPGK

SEQ ID NO: 13 - protein, 232 aa, Homo sapiens
EPKSCDKTHTCPPCPAPELLGGPSVFLFPPKPKDTLMISRTPEVTCVVVDVSHEDPEVKFNWYVDGVEVHNAKTKPREEQYNSTYRVVSVLTVLHQDWLNGKEYKCKVSNKALPAPIEKTISKAKGQPREPQVYTLPPSREEMTKNQVSLTCLVKGFYPSDIAVEWESNGQPENNYKTTPPVLDSDGSFFLYSKLTVDKSRWQQGNVFSCSVMHEGLHNHYTQKSLSLSPGK

SEQ ID NO: 14 - protein, 228 aa, Homo sapiens
ERKCCVECPPCPAPPVAGPSVFLFPPKPKDTLMISRTPEVTCVVVDVSHEDPEVQFNWYVDGVEVHNAKTKPREEQYNSTYRVVSVLTVLHQDWLNGKEYKCKVSNKALPAPIEKTISKTKGQPREPQVYTLPPSREEMTKNQVSLTCLVKGFYPSDIAVEWESNGQPENNYKTTPPMLDSDGSFFLYSKLTVDKSRWQQGNVFSCSVMHEALHNHYTQKSLSLSPGK

SEQ ID NO: 15 - protein, 279 aa, Homo sapiens
ELKTPLGDTTHTCPRCPEPKSCDTPPPCPRCPEPKSCDTPPPCPRCPEPKSCDTPPPCPRCPAPELLGGPSVFLFPPKPKDTLMISRTPEVTCVVVDVSHEDPEVQFKWYVDGVEVHNAKTKPREEQYNSTFRVVSVLTVLHQDWLNGKEYKCKVSNKALPAPIEKTISKTKGQPREPQVYTLPPSREEMTKNQVSLTCLVKGFYPSDIAVEWESSGQPENNYNTTPPMLDSDGSFFLYSKLTVDKSRWQQGNIFSCSVMHEALHNRFTQKSLSLSPGK

SEQ ID NO: 16 - protein, 228 aa, Homo sapiens
ESKYGPPCPSPAPEFLGGPSVFLFPPKPKDTLMISRTPEVTCVVVDVSQEDPEVQFNWYVDGMEVHNAKTKPREEQFNSTFRVVSVLTVVHQDWLNGKEYKCKVSNKGLPAPIEKTISKAKGQPREPQVYTLPPSQEEMTKNQVSLTCLVKGFYPSDIAVEWESNGQPENNYKTTPPVLDSDGSFFLYSRLTVDKSRWQEGNVFSCSVMHEALHNHYTQKSLSLSLGK